European Patent Specification EP 3 250 192 B1, published October 8, 2025. Title: COMPOSITIONS AND METHODS OF USING TYROSINE KINASE INHIBITORS. Applicant: Yale University Bennett, Anton Yi, Jae-Sung. The sequence listing filed with the application follows.

SEQUENCE LISTING (14 sequences)

SEQ ID NO: 1 - DNA, 21 bp, Artificial Sequence
  Synthetic sequence
accgcagctaggaataatgga

SEQ ID NO: 2 - DNA, 19 bp, Artificial Sequence
  Synthetic sequence
accaaaagccttgactccg

SEQ ID NO: 3 - DNA, 25 bp, Artificial Sequence
  Synthetic sequence
cctggaggagaagatgccggtagaa

SEQ ID NO: 4 - DNA, 24 bp, Artificial Sequence
  Synthetic sequence
ccccagtccagggaggcacctcgg

SEQ ID NO: 5 - DNA, 26 bp, Artificial Sequence
  Synthetic sequence
cacttcaaaggtggtcccagagctgc

SEQ ID NO: 6 - DNA, 23 bp, Artificial Sequence
  Synthetic sequence
gaccggatcggatccgtcagtcg

SEQ ID NO: 7 - DNA, 22 bp, Artificial Sequence
  Synthetic sequence
gtcccggacactggaccaggcc

SEQ ID NO: 8 - DNA, 27 bp, Artificial Sequence
  Synthetic sequence
ctccttttcttccagttgcctagccaa

SEQ ID NO: 9 - DNA, 25 bp, Artificial Sequence
  Synthetic sequence
gagcaaggccgaggagacgcagcgt

SEQ ID NO: 10 - DNA, 26 bp, Artificial Sequence
  Synthetic sequence
gagcctccttctcgtccagctgccgg

SEQ ID NO: 11 - DNA, 20 bp, Artificial Sequence
  Synthetic sequence
aggtcttcctggagctgatg

SEQ ID NO: 12 - DNA, 20 bp, Artificial Sequence
  Synthetic sequence
acccacagggccttctttac

SEQ ID NO: 13 - DNA, 24 bp, Artificial Sequence
  Synthetic sequence
acagcaaattcacttacacagttc

SEQ ID NO: 14 - DNA, 19 bp, Artificial Sequence
  Synthetic sequence
ctcattgccttgcgtgttt